European Patent Application EP 4 227 398 A1, published August 16, 2023. Title: Method for detecting target substance, fluid device and kit. Applicant: RIKEN. The sequence listing filed with the application follows.

SEQUENCE LISTING (5 sequences)

SEQ ID NO: 1 - DNA, 20 bp, Artificial Sequence
  Synthesyzed oligonucleotide
gccaagcgcacctaatttcc

SEQ ID NO: 2 - RNA, 40 nt, Artificial Sequence
  Synthesyzed oligonucleotide
aauuucuacuaaguguagauggaaauuaggugcgcuuggc

SEQ ID NO: 3 - RNA, 28 nt, Artificial Sequence
  Synthesyzed oligonucleotide
auggauuacuugguagaacagcaaucua

SEQ ID NO: 4 - RNA, 64 nt, Artificial Sequence
  Synthesyzed oligonucleotide
gauuuagacuaccccaaaaacgaaggggacuaaaacuagauugcuguucuaccaaguaauccau

SEQ ID NO: 5 - RNA, 120 nt, Artificial Sequence
  Synthesyzed oligonucleotide
gggggccagugaauucgagcucgguacccggggauccucuagaaauauggauuacuugguagaacagcaaucuacucgaccugcaggcaugcaagcuuggcguaaucauggucauagcug